European Patent Specification EP 4 504 967 B1, published July 2, 2025. Title: METHOD FOR DETECTING TARGET NUCLEIC ACID MOLECULES. Applicant: READILY AB. Application SE. The sequence listing filed with the application follows.

SEQUENCE LISTING (11 sequences)

SEQ ID NO: 1 - DNA, 77 bp, synthetic construct
  source 1..77: mol_type = other DNA
tgtactcaccggttcctattacgccgcaacagcacgcatacttgagctcatatgtggtattgtcctggcaattccgg

SEQ ID NO: 2 - DNA, 77 bp, synthetic construct
  source 1..77: mol_type = other DNA
ccggttccgcagaccctattacgccgcaacagcacgcatacttgagctcatatgtggtattgattccggagtactca

SEQ ID NO: 3 - DNA, 77 bp, synthetic construct
  source 1..77: mol_type = other DNA
cagcacgcaccggttctattacgccgcaacagcacgcatacttgagctcatatgtggtattgctcagcggctataat

SEQ ID NO: 4 - DNA, 33 bp, synthetic construct
  source 1..33: mol_type = other DNA
gaaccggtgagtacaccggaattgccaggacga

SEQ ID NO: 5 - DNA, 33 bp, synthetic construct
  source 1..33: mol_type = other DNA
ggtctgcggaaccggtgagtacaccggaattac

SEQ ID NO: 6 - DNA, 40 bp, synthetic construct
  source 1..40: mol_type = other DNA
gcggaaccggtgcgtgctgattatagccgctgagtacacc

SEQ ID NO: 7 - DNA, 12 bp, synthetic construct
  source 1..12: mol_type = other DNA
cgagtatacacc

SEQ ID NO: 8 - DNA, 65 bp, synthetic construct
  source 1..65: mol_type = other DNA
tgtactcaccggttcctattacgccgcaacagcacgcatacttgatattgtcctggcaattccgg

SEQ ID NO: 9 - DNA, 65 bp, synthetic construct
  source 1..65: mol_type = other DNA
ccggttccgcagaccctattacgccgcaacagcacgcatacttgatattgattccggagtactca

SEQ ID NO: 10 - DNA, 65 bp, synthetic construct
  source 1..65: mol_type = other DNA
cagcacgcaccggttctattacgccgcaacagcacgcatacttgatattgctcagcggctataat

SEQ ID NO: 11 - DNA, 13 bp, synthetic construct
  source 1..13: mol_type = other DNA
ggtgtatatctcg